European Patent Specification EP 3 660 045 B1, published August 7, 2024. Title: Polypeptide, process for the production thereof and use thereof. Applicant: Shanxi jinbo Bio-pharmaceutical Co,Ltd. The sequence listing filed with the application follows.

SEQUENCE LISTING (12 sequences)

SEQ ID NO: 1 - protein, 30 aa, Homo sapiens
GERGAPGFRGPAGPNGIPGEKGPAGERGAP

SEQ ID NO: 2 - protein, 10 aa, artifical sequence
  the C terminal sequence
GPPGPCCGGG

SEQ ID NO: 3 - protein, 480 aa, artifical sequence
  TE16C
GERGAPGFRGPAGPNGIPGEKGPAGERGAPGERGAPGFRGPAGPNGIPGEKGPAGERGAPGERGAPGFRGPAGPNGIPGEKGPAGERGAPGERGAPGFRGPAGPNGIPGEKGPAGERGAPGERGAPGFRGPAGPNGIPGEKGPAGERGAPGERGAPGFRGPAGPNGIPGEKGPAGERGAPGERGAPGFRGPAGPNGIPGEKGPAGERGAPGERGAPGFRGPAGPNGIPGEKGPAGERGAPGERGAPGFRGPAGPNGIPGEKGPAGERGAPGERGAPGFRGPAGPNGIPGEKGPAGERGAPGERGAPGFRGPAGPNGIPGEKGPAGERGAPGERGAPGFRGPAGPNGIPGEKGPAGERGAPGERGAPGFRGPAGPNGIPGEKGPAGERGAPGERGAPGFRGPAGPNGIPGEKGPAGERGAPGERGAPGFRGPAGPNGIPGEKGPAGERGAPGERGAPGFRGPAGPNGIPGEKGPAGERGAP

SEQ ID NO: 4 - protein, 6 aa, artifical sequence
  the N terminal sequence
ENLYFQ

SEQ ID NO: 5 - protein, 486 aa, artifical sequence
  TE16C having the N terminal sequence
ENLYFQGERGAPGFRGPAGPNGIPGEKGPAGERGAPGERGAPGFRGPAGPNGIPGEKGPAGERGAPGERGAPGFRGPAGPNGIPGEKGPAGERGAPGERGAPGFRGPAGPNGIPGEKGPAGERGAPGERGAPGFRGPAGPNGIPGEKGPAGERGAPGERGAPGFRGPAGPNGIPGEKGPAGERGAPGERGAPGFRGPAGPNGIPGEKGPAGERGAPGERGAPGFRGPAGPNGIPGEKGPAGERGAPGERGAPGFRGPAGPNGIPGEKGPAGERGAPGERGAPGFRGPAGPNGIPGEKGPAGERGAPGERGAPGFRGPAGPNGIPGEKGPAGERGAPGERGAPGFRGPAGPNGIPGEKGPAGERGAPGERGAPGFRGPAGPNGIPGEKGPAGERGAPGERGAPGFRGPAGPNGIPGEKGPAGERGAPGERGAPGFRGPAGPNGIPGEKGPAGERGAPGERGAPGFRGPAGPNGIPGEKGPAGERGAP

SEQ ID NO: 6 - protein, 501 aa, artifical sequence
  HC16
GERGAPGFRGPAGPNGIPGEKGPAGERGAPGERGAPGFRGPAGPNGIPGEKGPAGERGAPGERGAPGFRGPAGPNGIPGEKGPAGERGAPGERGAPGFRGPAGPNGIPGEKGPAGERGAPRSGERGAPGFRGPAGPNGIPGEKGPAGERGAPGERGAPGFRGPAGPNGIPGEKGPAGERGAPGERGAPGFRGPAGPNGIPGEKGPAGERGAPGERGAPGFRGPAGPNGIPGEKGPAGERGAPRSGERGAPGFRGPAGPNGIPGEKGPAGERGAPGERGAPGFRGPAGPNGIPGEKGPAGERGAPGERGAPGFRGPAGPNGIPGEKGPAGERGAPGERGAPGFRGPAGPNGIPGEKGPAGERGAPRSGERGAPGFRGPAGPNGIPGEKGPAGERGAPGERGAPGFRGPAGPNGIPGEKGPAGERGAPGERGAPGFRGPAGPNGIPGEKGPAGERGAPGERGAPGFRGPAGPNGIPGEKGPAGERGAPRSPEFGPPGPCCGGG

SEQ ID NO: 7 - DNA, 1458 bp, artifical sequence
  TE16C having the N terminal sequence
gaaaacctgtatttccagggtgaacgtggtgcaccaggttttcgtggtccggcaggtccgaatggaattccgggtgagaaaggaccggctggtgagcgtggtgcgccgggtgaacgtggagcgcctggttttcgtggcccagcaggtccgaacggtattcctggtgaaaaaggtccggcgggagagcgtggtgcaccgggtgaacgcggtgcaccgggatttcgtggtccagcaggaccgaatggtatccctggtgaaaaaggaccggcaggtgagcgtggagcgccaggtgaacgtggcgcaccgggttttcgtggaccggcaggcccgaatggtattccgggtgaaaaaggcccggcaggtgaacgtggtgccccgggtgaacgtggtgcgcctggatttcgtggcccggcaggaccgaacggtatccctggagaaaaaggtcctgcaggtgagcgcggtgcgccgggcgagcgtggtgcccctggttttcgcggtccggcaggccctaatggtattcctggagaaaaaggccctgcaggtgaacgcggagcaccgggtgagcgtggcgcacctggttttcgtggtcctgcaggcccgaacggtattccgggcgaaaaaggtccagcaggtgaacgtggtgctccgggtgaacgtggtgcacctggatttcgcggtcctgctggtccgaatggtattccaggtgaaaaaggtccggcaggagagcgtggagcaccgggagaacgtggtgcaccgggctttcgtggtccggccggtcctaacggtatcccaggtgaaaaaggtccggccggcgagcgtggcgcccctggtgagcgtggtgctcctggttttcgtggtccggctggtccgaacggaattcctggtgagaaaggtccggctggcgaacgtggtgcaccgggtgaacgtggtgcaccgggtttccgtggtccggcgggtcctaatggtatcccgggtgaaaaaggtccggcaggtgaacgtggtgcaccgggtgaacgtggtgcaccgggttttcgcggaccggcaggacctaatggtattccgggagaaaaaggacctgcgggtgaacgtggtgcaccgggtgaacgtggtgcaccgggttttcgtggtccggcaggtcctaatggaattcctggagagaaaggacctgcaggtgaacgtggtgcaccgggtgaacgtggtgcaccgggttttcgtggtccggcaggtccaaatggtattccgggtgaaaaaggtccggcaggtgaacgtggtgcaccgggtgaacgtggtgcaccgggttttcgtggtccggcaggtccgaatggcattcctggtgaaaaaggtccggcaggtgaacgtggtgcaccgggtgaacgtggtgcaccgggttttcgtggtccggcaggtccgaatggtattccgggtgaaaaaggtccggcaggtgaacgtggtgcaccg

SEQ ID NO: 8 - DNA, 1503 bp, artifical sequence
  HC16
ggcgagcgtggtgcacctggttttcgtggccctgcaggcccgaatggcatcccgggtgaaaaaggcccggcaggcgaacgtggcgcccctggtgaacgcggcgcacctggtttccgtggcccggcaggtcctaacggtatcccgggcgaaaagggtcctgcaggcgagcgtggcgccccgggtgaacgcggtgcccctggctttcgcggtcctgccggccctaacggcattccgggtgagaaaggtcctgccggtgagcgcggtgcccctggtgagcgcggcgcaccgggctttcgtggcccggccggtcctaatggtattcctggcgagaagggtccggcaggtgaacgcggtgcacctagatccggcgagcgtggtgcacctggttttcgtggccctgcaggcccgaatggcatcccgggtgaaaaaggcccggcaggcgaacgtggcgcccctggtgaacgcggcgcacctggtttccgtggcccggcaggtcctaacggtatcccgggcgaaaagggtcctgcaggcgagcgtggcgccccgggtgaacgcggtgcccctggctttcgcggtcctgccggccctaacggcattccgggtgagaaaggtcctgccggtgagcgcggtgcccctggtgagcgcggcgcaccgggctttcgtggcccggccggtcctaatggtattcctggcgagaagggtccggcaggtgaacgcggtgcacctagatccggcgagcgtggtgcacctggttttcgtggccctgcaggcccgaatggcatcccgggtgaaaaaggcccggcaggcgaacgtggcgcccctggtgaacgcggcgcacctggtttccgtggcccggcaggtcctaacggtatcccgggcgaaaagggtcctgcaggcgagcgtggcgccccgggtgaacgcggtgcccctggctttcgcggtcctgccggccctaacggcattccgggtgagaaaggtcctgccggtgagcgcggtgcccctggtgagcgcggcgcaccgggctttcgtggcccggccggtcctaatggtattcctggcgagaagggtccggcaggtgaacgcggtgcacctagatccggcgagcgtggtgcacctggttttcgtggccctgcaggcccgaatggcatcccgggtgaaaaaggcccggcaggcgaacgtggcgcccctggtgaacgcggcgcacctggtttccgtggcccggcaggtcctaacggtatcccgggcgaaaagggtcctgcaggcgagcgtggcgccccgggtgaacgcggtgcccctggctttcgcggtcctgccggccctaacggcattccgggtgagaaaggtcctgccggtgagcgcggtgcccctggtgagcgcggcgcaccgggctttcgtggcccggccggtcctaatggtattcctggcgagaagggtccggcaggtgaacgcggtgcacctagatctccggaattcggcccgcctggtccttgttgtggcggcggc

SEQ ID NO: 9 - protein, 490 aa, artifical sequence
  T16a
GERGAPGFRGPAGPNGIPGEKGPAGERGAPGERGAPGFRGPAGPNGIPGEKGPAGERGAPGERGAPGFRGPAGPNGIPGEKGPAGERGAPGERGAPGFRGPAGPNGIPGEKGPAGERGAPGERGAPGFRGPAGPNGIPGEKGPAGERGAPGERGAPGFRGPAGPNGIPGEKGPAGERGAPGERGAPGFRGPAGPNGIPGEKGPAGERGAPGERGAPGFRGPAGPNGIPGEKGPAGERGAPGERGAPGFRGPAGPNGIPGEKGPAGERGAPGERGAPGFRGPAGPNGIPGEKGPAGERGAPGERGAPGFRGPAGPNGIPGEKGPAGERGAPGERGAPGFRGPAGPNGIPGEKGPAGERGAPGERGAPGFRGPAGPNGIPGEKGPAGERGAPGERGAPGFRGPAGPNGIPGEKGPAGERGAPGERGAPGFRGPAGPNGIPGEKGPAGERGAPGERGAPGFRGPAGPNGIPGEKGPAGERGAPGPPGPCCGGG

SEQ ID NO: 10 - DNA, 1470 bp, artifical sequence
  T16a
ggtgaacgtggtgcaccaggttttcgtggtccggcaggtccgaatggaattccgggtgagaaaggaccggctggtgagcgtggtgcgccgggtgaacgtggagcgcctggttttcgtggcccagcaggtccgaacggtattcctggtgaaaaaggtccggcgggagagcgtggtgcaccgggtgaacgcggtgcaccgggatttcgtggtccagcaggaccgaatggtatccctggtgaaaaaggaccggcaggtgagcgtggagcgccaggtgaacgtggcgcaccgggttttcgtggaccggcaggcccgaatggtattccgggtgaaaaaggcccggcaggtgaacgtggtgccccgggtgaacgtggtgcgcctggatttcgtggcccggcaggaccgaacggtatccctggagaaaaaggtcctgcaggtgagcgcggtgcgccgggcgagcgtggtgcccctggttttcgcggtccggcaggccctaatggtattcctggagaaaaaggccctgcaggtgaacgcggagcaccgggtgagcgtggcgcacctggttttcgtggtcctgcaggcccgaacggtattccgggcgaaaaaggtccagcaggtgaacgtggtgctccgggtgaacgtggtgcacctggatttcgcggtcctgctggtccgaatggtattccaggtgaaaaaggtccggcaggagagcgtggagcaccgggagaacgtggtgcaccgggctttcgtggtccggccggtcctaacggtatcccaggtgaaaaaggtccggccggcgagcgtggcgcccctggtgagcgtggtgctcctggttttcgtggtccggctggtccgaacggaattcctggtgagaaaggtccggctggcgaacgtggtgcaccgggtgaacgtggtgcaccgggtttccgtggtccggcgggtcctaatggtatcccgggtgaaaaaggtccggcaggtgaacgtggtgcaccgggtgaacgtggtgcaccgggttttcgcggaccggcaggacctaatggtattccgggagaaaaaggacctgcgggtgaacgtggtgcaccgggtgaacgtggtgcaccgggttttcgtggtccggcaggtcctaatggaattcctggagagaaaggacctgcaggtgaacgtggtgcaccgggtgaacgtggtgcaccgggttttcgtggtccggcaggtccaaatggtattccgggtgaaaaaggtccggcaggtgaacgtggtgcaccgggtgaacgtggtgcaccgggttttcgtggtccggcaggtccgaatggcattcctggtgaaaaaggtccggcaggtgaacgtggtgcaccgggtgaacgtggtgcaccgggttttcgtggtccggcaggtccgaatggtattccgggtgaaaaaggtccggcaggtgaacgtggtgcaccgggcccgcctggtccttgttgtggcggcggc

SEQ ID NO: 11 - protein, 486 aa, artifical sequence
  T16b
GERGAPGFRGPAGPNGIPGEKGPAGERGAPGERGAPGFRGPAGPNGIPGEKGPAGERGAPGERGAPGFRGPAGPNGIPGEKGPAGERGAPGERGAPGFRGPAGPNGIPGEKGPAGERGAPRSGERGAPGFRGPAGPNGIPGEKGPAGERGAPGERGAPGFRGPAGPNGIPGEKGPAGERGAPGERGAPGFRGPAGPNGIPGEKGPAGERGAPGERGAPGFRGPAGPNGIPGEKGPAGERGAPRSGERGAPGFRGPAGPNGIPGEKGPAGERGAPGERGAPGFRGPAGPNGIPGEKGPAGERGAPGERGAPGFRGPAGPNGIPGEKGPAGERGAPGERGAPGFRGPAGPNGIPGEKGPAGERGAPRSGERGAPGFRGPAGPNGIPGEKGPAGERGAPGERGAPGFRGPAGPNGIPGEKGPAGERGAPGERGAPGFRGPAGPNGIPGEKGPAGERGAPGERGAPGFRGPAGPNGIPGEKGPAGERGAP

SEQ ID NO: 12 - DNA, 1458 bp, artifical sequence
  T16b
ggcgagcgtggtgcacctggttttcgtggccctgcaggcccgaatggcatcccgggtgaaaaaggcccggcaggcgaacgtggcgcccctggtgaacgcggcgcacctggtttccgtggcccggcaggtcctaacggtatcccgggcgaaaagggtcctgcaggcgagcgtggcgccccgggtgaacgcggtgcccctggctttcgcggtcctgccggccctaacggcattccgggtgagaaaggtcctgccggtgagcgcggtgcccctggtgagcgcggcgcaccgggctttcgtggcccggccggtcctaatggtattcctggcgagaagggtccggcaggtgaacgcggtgcacctagatccggcgagcgtggtgcacctggttttcgtggccctgcaggcccgaatggcatcccgggtgaaaaaggcccggcaggcgaacgtggcgcccctggtgaacgcggcgcacctggtttccgtggcccggcaggtcctaacggtatcccgggcgaaaagggtcctgcaggcgagcgtggcgccccgggtgaacgcggtgcccctggctttcgcggtcctgccggccctaacggcattccgggtgagaaaggtcctgccggtgagcgcggtgcccctggtgagcgcggcgcaccgggctttcgtggcccggccggtcctaatggtattcctggcgagaagggtccggcaggtgaacgcggtgcacctagatccggcgagcgtggtgcacctggttttcgtggccctgcaggcccgaatggcatcccgggtgaaaaaggcccggcaggcgaacgtggcgcccctggtgaacgcggcgcacctggtttccgtggcccggcaggtcctaacggtatcccgggcgaaaagggtcctgcaggcgagcgtggcgccccgggtgaacgcggtgcccctggctttcgcggtcctgccggccctaacggcattccgggtgagaaaggtcctgccggtgagcgcggtgcccctggtgagcgcggcgcaccgggctttcgtggcccggccggtcctaatggtattcctggcgagaagggtccggcaggtgaacgcggtgcacctagatccggcgagcgtggtgcacctggttttcgtggccctgcaggcccgaatggcatcccgggtgaaaaaggcccggcaggcgaacgtggcgcccctggtgaacgcggcgcacctggtttccgtggcccggcaggtcctaacggtatcccgggcgaaaagggtcctgcaggcgagcgtggcgccccgggtgaacgcggtgcccctggctttcgcggtcctgccggccctaacggcattccgggtgagaaaggtcctgccggtgagcgcggtgcccctggtgagcgcggcgcaccgggctttcgtggcccggccggtcctaatggtattcctggcgagaagggtccggcaggtgaacgcggtgcacct